European Patent Specification EP 3 448 409 B1, published December 3, 2025. Title: Treatment of liver, biliary tract and pancreatic disorders. Applicant: Defensin Therapeutics ApS. The sequence listing filed with the application follows.

SEQUENCE LISTING (17 sequences)

SEQ ID NO: 1 - protein, 40 aa, Bos taurus
GVGNPVSCVRNKGICVPIRCPGSMKQIGTCVGRAVKCCRK

SEQ ID NO: 2 - protein, 34 aa, Gallus gallus
LFCKGGSCHFGGCPSHLIKVGSCFRSCCKWPWNA

SEQ ID NO: 3 - protein, 44 aa, Pongo pygmaeus
VFGDISNPVTCLRSGAICHPGFCPRRYKHIGTCGLSVIKCCKKP

SEQ ID NO: 4 - protein, 36 aa, Homo sapiens
DHYNCVSSGGQCLYSACPIFTKIQGTCYRGKAKCCK

SEQ ID NO: 5 - protein, 41 aa, Homo sapiens
GIGDPVTCLKSGAICHPVFCPRRYKQIGTCGLPGTKCCKKP

SEQ ID NO: 6 - protein, 45 aa, Homo sapiens
GIINTLQKYYCRVRGGRCAVLSCLPKEEQIGKCSTRGRKCCRRKK

SEQ ID NO: 7 - protein, 37 aa, Homo sapiens
ELDRICGYGTARCRKKCRSQEYRIGRCPNTYACCLRK

SEQ ID NO: 8 - protein, 32 aa, Homo sapiens
ATCYCRTGRCATRESLSGVCEISGRLYRLCCR

SEQ ID NO: 9 - protein, 32 aa, Homo sapiens
AFTCHCRRSCYSTEYSYGTCTVMGINHRFCCL

SEQ ID NO: 10 - protein, 41 aa, Pan troglodytes
GISDPVTCLKSGAICHPVFCPRRYKQIGTCGLPGTKCCKKP

SEQ ID NO: 11 - protein, 41 aa, Macaca mulatta
GIGDPVTCLKNGAICHPVFCPRRYKQIGTCGLPGTKCCKKP

SEQ ID NO: 12 - protein, 40 aa, Mus musculus
KINNPVSCLRKGGRCWNRCIGNTRQIGSCGVPFLKCCKRK

SEQ ID NO: 13 - protein, 40 aa, Equus caballus
GIGNPISCARNRGVCIPIGCLPGMKQIGTCGLPGTKCCRK

SEQ ID NO: 14 - protein, 40 aa, Sus scrofa
NIGNSVSCLRNKGVCMPGKCAPKMKQIGTCGMPQVKCCKR

SEQ ID NO: 15 - protein, 40 aa, Capra aegagrus
GIINHRSCYRNKGVCAPARCPRNMRQIGTCHGPPVKCCRK

SEQ ID NO: 16 - protein, 37 aa, Homo sapiens
LLGDFFRKSKEKIGKEFKRIVQRIKDFLRNLVPRTES

SEQ ID NO: 17 - protein, 37 aa, Homo sapiens
PVTCLKSGAICHPVFCPRRYKQIGTCGLPGTKCCKKP